European Patent Application EP 4 497 822 A1, published January 29, 2025. Title: 制御性Ｔ細胞の製造方法. Applicant: 国立大学法人京都大学. The sequence listing filed with the application follows.

SEQUENCE LISTING (9 sequences)

SEQ ID NO: 1 - DNA, 1191 bp, Homo sapiens
  source 1..1191: mol_type = other DNA
atgcccaaccccaggcctggcaagccctcggccccttccttggcccttggcccatccccaggagcctcgcccagctggagggctgcacccaaagcctcagacctgctgggggcccggggcccagggggaaccttccagggccgagatcttcgaggcggggcccatgcctcctcttcttccttgaaccccatgccaccatcgcagctgcagctctcaacggtggatgcccacgcccggacccctgtgctgcaggtgcaccccctggagagcccagccatgatcagcctcacaccacccaccaccgccactggggtcttctccctcaaggcccggcctggcctcccacctgggatcaacgtggccagcctggaatgggtgtccagggagccggcactgctctgcaccttcccaaatcccagtgcacccaggaaggacagcaccctttcggctgtgccccagagctcctacccactgctggcaaatggtgtctgcaagtggcccggatgtgagaaggtcttcgaagagccagaggacttcctcaagcactgccaggcggaccatcttctggatgagaagggcagggcacaatgtctcctccagagagagatggtacagtctctggagcagcagctggtgctggagaaggagaagctgagtgccatgcaggcccacctggctgggaaaatggcactgaccaaggcttcatctgtggcatcatccgacaagggctcctgctgcatcgtagctgctggcagccaaggccctgtcgtcccagcctggtctggcccccgggaggcccctgacagcctgtttgctgtccggaggcacctgtggggtagccatggaaacagcacattcccagagttcctccacaacatggactacttcaagttccacaacatgcgaccccctttcacctacgccacgctcatccgctgggccatcctggaggctccagagaagcagcggacactcaatgagatctaccactggttcacacgcatgtttgccttcttcagaaaccatcctgccacctggaagaacgccatccgccacaacctgagtctgcacaagtgctttgtgcgggtggagagcgagaagggggctgtgtggaccgtggatgagctggagttccgcaagaaacggagccagaggcccagcaggtgttccaaccctacacctggcccctga

SEQ ID NO: 2 - DNA, 1296 bp, Homo sapiens
  source 1..1296: mol_type = other DNA
atgcccaaccccaggcctggcaagccctcggccccttccttggcccttggcccatccccaggagcctcgcccagctggagggctgcacccaaagcctcagacctgctgggggcccggggcccagggggaaccttccagggccgagatcttcgaggcggggcccatgcctcctcttcttccttgaaccccatgccaccatcgcagctgcagctgcccacactgcccctagtcatggtggcaccctccggggcacggctgggccccttgccccacttacaggcactcctccaggacaggccacatttcatgcaccagctctcaacggtggatgcccacgcccggacccctgtgctgcaggtgcaccccctggagagcccagccatgatcagcctcacaccacccaccaccgccactggggtcttctccctcaaggcccggcctggcctcccacctgggatcaacgtggccagcctggaatgggtgtccagggagccggcactgctctgcaccttcccaaatcccagtgcacccaggaaggacagcaccctttcggctgtgccccagagctcctacccactgctggcaaatggtgtctgcaagtggcccggatgtgagaaggtcttcgaagagccagaggacttcctcaagcactgccaggcggaccatcttctggatgagaagggcagggcacaatgtctcctccagagagagatggtacagtctctggagcagcagctggtgctggagaaggagaagctgagtgccatgcaggcccacctggctgggaaaatggcactgaccaaggcttcatctgtggcatcatccgacaagggctcctgctgcatcgtagctgctggcagccaaggccctgtcgtcccagcctggtctggcccccgggaggcccctgacagcctgtttgctgtccggaggcacctgtggggtagccatggaaacagcacattcccagagttcctccacaacatggactacttcaagttccacaacatgcgaccccctttcacctacgccacgctcatccgctgggccatcctggaggctccagagaagcagcggacactcaatgagatctaccactggttcacacgcatgtttgccttcttcagaaaccatcctgccacctggaagaacgccatccgccacaacctgagtctgcacaagtgctttgtgcgggtggagagcgagaagggggctgtgtggaccgtggatgagctggagttccgcaagaaacggagccagaggcccagcaggtgttccaaccctacacctggcccctga

SEQ ID NO: 3 - protein, 396 aa, Homo sapiens
MPNPRPGKPSAPSLALGPSPGASPSWRAAPKASDLLGARGPGGTFQGRDLRGGAHASSSSLNPMPPSQLQLSTVDAHARTPVLQVHPLESPAMISLTPPTTATGVFSLKARPGLPPGINVASLEWVSREPALLCTFPNPSAPRKDSTLSAVPQSSYPLLANGVCKWPGCEKVFEEPEDFLKHCQADHLLDEKGRAQCLLQREMVQSLEQQLVLEKEKLSAMQAHLAGKMALTKASSVASSDKGSCCIVAAGSQGPVVPAWSGPREAPDSLFAVRRHLWGSHGNSTFPEFLHNMDYFKFHNMRPPFTYATLIRWAILEAPEKQRTLNEIYHWFTRMFAFFRNHPATWKNAIRHNLSLHKCFVRVESEKGAVWTVDELEFRKKRSQRPSRCSNPTPGP

SEQ ID NO: 4 - protein, 431 aa, Homo sapiens
MPNPRPGKPSAPSLALGPSPGASPSWRAAPKASDLLGARGPGGTFQGRDLRGGAHASSSSLNPMPPSQLQLPTLPLVMVAPSGARLGPLPHLQALLQDRPHFMHQLSTVDAHARTPVLQVHPLESPAMISLTPPTTATGVFSLKARPGLPPGINVASLEWVSREPALLCTFPNPSAPRKDSTLSAVPQSSYPLLANGVCKWPGCEKVFEEPEDFLKHCQADHLLDEKGRAQCLLQREMVQSLEQQLVLEKEKLSAMQAHLAGKMALTKASSVASSDKGSCCIVAAGSQGPVVPAWSGPREAPDSLFAVRRHLWGSHGNSTFPEFLHNMDYFKFHNMRPPFTYATLIRWAILEAPEKQRTLNEIYHWFTRMFAFFRNHPATWKNAIRHNLSLHKCFVRVESEKGAVWTVDELEFRKKRSQRPSRCSNPTPGP

SEQ ID NO: 5 - DNA, 238 bp, Homo sapiens
  source 1..238: mol_type = other DNA
taggttagtctttttttctgtggcttctgtctctggttttgtgcttagaaagtcctttcctacttgaaaatgagataaatgttcacctatgttggcttctagtctcttttatggcttcattttttccatttactatagaggttaagagtgtgggtactggagccagactgtctgggacaaacccagcgtcaccccaagccctatgtgtgatttttagccaggcacttaacctctccat

SEQ ID NO: 6 - DNA, 360 bp, Homo sapiens
  source 1..360: mol_type = other DNA
ccaagaagggccaggtcttcagagctaggggcttgtcatagtggccagatggacatcacctaccacatccaccagcacccatgtcaccccacctgggccaagcctgctgcaggacagggcagccagttctcggaacgaaacctgtggggtggggtatctgccctcttctcttcctccgtggtgtcgatgaagcccggcgcatccggccgccatgacgtcaatggcggaaaaatctgggcaagtcgggggctgtgacaacagggcccagatgcagaccccgatatgaaaacataatctgtgtcccagaaacatcccccattcagcttctgagaaacccagtcagaaagggacgtcccaaca

SEQ ID NO: 7 - DNA, 218 bp, Homo sapiens
  source 1..218: mol_type = other DNA
gaggccctgggcccaggatggggcaggcagggtggggtacctggacctacaggtgccgacctttactgtggcactgggcgggaggggggctggctggggcacaggaagtggtttctgggtcccaggcaagtctgtgacttatgcagatgttgcagggccaagaaaatccccacctgccaggcctcagagattggaggctctccccgacctcccaatcc

SEQ ID NO: 8 - DNA, 383 bp, Homo sapiens
  source 1..383: mol_type = other DNA
tcccatccacacatagagcttcagattctctttctttccccagagaccctcaaatatcctctcactcacagaatggtgtctctgcctgcctcgggttggccctgtgatttattttagttcttttcccttgttttttttttttcaaactctatacacttttgttttaaaaactgtggtttctcatgagccctattatctcattgatacctctcacctctgtggtgaggggaagaaatcatattttcagatgactcgtaaagggcaaagaaaaaaacccaaaatttcaaaatttccgtttaagtctcataatcaagaaaaggagaaacacagagagagagaaaaaaaaaactatgagaacccctccccaccccgtgattatcagc

SEQ ID NO: 9 - DNA, 1632 bp, synthetic construct
  source 1..1632: mol_type = other DNA
atggacttccaggtgcagatcttcagcttcctgctgatcagcgccagcgtgatcatgagccgcgctagccaggtgcagctgcagcagagcggccccgagctggtgaagcccggcgccagcgtgaagatgagctgcaaggccagcggctacaccttcaccagctaccacatccagtgggtgaagcagcgccccggccagggcctggagtggatcggctggatctaccccggcgacggcagcacccagtacaacgagaagttcaagggcaagaccaccctgaccgccgacaagagcagcagcaccgcctacatgctgctgagcagcctgaccagcgaggacagcgccatctacttctgcgcccgcgagggcacctactacgccatggactactggggccagggcaccagcgtgaccgtgagcagcgtcgacagcagcggcggcggcggcagcggcggcggcggcagcggcggcggcggcagcactagtgacgtgctgatgacccagacccccctgagcctgcccgtgagcctgggcgaccaggtgagcatcagctgccgcagcagccagagcatcgtgcacagcaacggcaacacctacctggagtggtacctgcagaagcccggccagagccccaagctgctgatctacaaggtgagcaaccgcttcagcggcgtgcccgaccgcttcagcggcagcggcagcggcaccgacttcaccctgaagatcagccgcgtggaggccgaggacctgggcgtgtactactgcttccagggcagccacgtgccccgcaccttcggcggcggcaccaagctggagatcaagctcgagcagaagctgatcagcgaggaggacctgaaccggatccgtggggtcaccgtctcttcagcgctgagcaactccatcatgtacttcagccacttcgtgccggtcttcctgccagcgaagcccaccacgacgccagcgccgcgaccaccaacaccggcgcccaccatcgcgtcgcagcccctgtccctgcgcccagaggcgtgccggccagcggcggggggcgcagtgcacacgagggggctggacccctttgggttttgggtgctggtggtggttggtggagtcctggcttgctatagcttgctagtaacagtggcctttattattttctgggtgaggagtaagaggagcaggctcctgcacagtgactacatgaacatgactccccgccgccccgggcccacccgcaagcattaccagccctatgccccaccacgcgacttcgcagcctatcgctccctcgagagagtgagagtgaagttcagcaggagcgcagacgcccccgcgtaccagcagggccagaaccagctctataacgagctcaatctaggacgaagagaggagtacgatgttttggacaagagacgtggccgggaccctgagatggggggaaagccgagaaggaagaaccctcaggaaggcctgtacaatgaactgcagaaagataagatggcggaggcctacagtgagattgggatgaaaggcgagcgccggaggggcaaggggcacgatggcctttaccagggtctcagtacagccaccaaggacacctacgacgcccttcacatgcaggccctgccccctcgc